European Patent Application EP 4 360 641 A1, published May 1, 2024. Title: USE OF MAZDUTIDE. Applicant: Innovent Biologics (Suzhou) Co., Ltd. The sequence listing filed with the application follows.

SEQUENCE LISTING (1 sequence)

SEQ ID NO: 1 - protein, 34 aa, Artificial Sequence
  OMX3 sequence
  MOD_RES (2)..(2): Xaa is Aib
  MOD_RES (20)..(20): Lys at position 20 is chemically modified by conjugating with ε-amino group of the K side chain via ([2-(2-amino-ethoxy)-ethoxy]-acetyl)2-(γGlu)1-CO-(CH 2)18-CO2H
  MOD_RES (34)..(34): Gly is amidated to a C-terminal primary amide
HXQGTFTSDYSKYLDEKKAKEFVEWLLEGGPSSG